European Patent Application EP 4 260 685 A1, published October 18, 2023. Title: Tobacco plant and tobacco product. Applicant: JAPAN TOBACCO INC. The sequence listing filed with the application follows.

SEQUENCE LISTING (25 sequences)

SEQ ID NO: 1 - DNA, 2715 bp, Nicotiana tabacum
  CDS (1)..(2715)
atggcggcatctgtcgaaaacaggcagttcagtcacatagaagccggtttatcccggtctttcaagcctcggtctgattccccggttcgtggctgcaacttccctccgcccaacagtactaatttccaaaagaaaccaaattccaccattttccttgattactcgtcgagtgaagacgacgatgatgatgacgaaaaaaatgagtaccttcaaatgatcaaaaaagggaattcagaattagagccatctgttcatgacagcagggacgaaggtaccgctgataactggattgaacgcaacttttccttgattcgtctcaccggaaagcatccatttaactccgaaccgccgttgaaccgtctcatgcaccacggttttatcacaccggtcccacttcattacgttcgtaaccatggaccggttcccaagggcacatgggatgactggaccgtggaagtcacgggactagtgaaacgtcctatgaaattcacaatggaccagttggttaacgaattcccttccagagaattgcccgttacgcttgtgtgtgctggcaaccgaaggaaagaacagaacatggttaaacaaaccattggtttcaactggggtgccgctgccgtttcaacaactgtatggcgcggggtacccctacgcgctttgttaaaacggtgcggtgtttttagcaagaataaaggggcgcttaatgtttgcttcgaaggagctgatgtcttgcccggaggcggtggttcaaagtatggaaccagcattaagaaggaatttgcaatggatccagcacgagatatcataatagcttacatgcagaacggagaaaaattggcacccgaccacgggtttccagtacgaatgataattccaggattcattggaggaagaatggtgaaatggataaagaggattatagtcaccacccaagaatcagacagctattatcatttcaaggacaatagagttcttcctccccatgttgatgctgaacttgcaaatactgaagcatggtggtacaagccagagtacatcatcaatgagctcaatattaactctgtcattacgacgccgtgtcatgaagaaattttgcctattaacgcctggacgactcagcgaccttacacgttgaggggctattcttattctggcggagggaaaaaagtaacgcgagtagaagtgaccttggatggaggagaaacatggcaagtttgcacactagatcacccagagaagcccaccaaatatggcaagtactggtgttggtgcttttggtcactcgaggttgaggtgttagacttgctcagtgccaaagaaattgctgttcgagcttgggatgagaccctcaatactcaacctgagaagcttatttggaatgtcatgggaatgatgaacaattgctggttccgagtaaagatgaatgtgtgcaagcctcacaagggagagattggaatagtgtttgaacacccgactcaacctggaaaccaatcaggtggatggatggcaaaggagaggcatttggagatatcagcagaggcacctccaacactaaagaagagtatctcaactccattcatgaacacagcttccaagatgtactccatgtcggaggtgaggaaacacagctctgctgactctgcttggatcatagtccatggtcatatctatgacgccacgcgtttcttgaaagatcaccccggtggttctgacagcattctcatcaatgctggcactgattgcactgaggaatttgatgcaattcattctgataaggctaagaagctattggaggaattcaggattggtgaactcataactactggttacacctctgactctcctggcaactccgtccatggatcttcttccttcagcagctttctagcacctattaaggaacttgttccagcgcagaggagtgtggccctcattccaagagagaaaatcccatgcaaactcatcgacaaacaatccatctcccctgatgttaggaaatttcgatttgcattgccctctgaggatcaagtcttgggcttgcctgttggtaaacacatcttcctctgtgccgttattgacgataagctctgcatgcgcgcctacacgcctactagcacgatcgatgaggtggggtacttcgagttggttgtcaagatatacttcaaaggaattcaccctaaattccccaatggggggcaaatgtcacaataccttgattctctccaattagggtcatttctcgacgtgaaaggtccattaggtcacattgaataccaaggaaagggcaatttcttagttcatggcaaacaaaagtttgccaagaagttggccatgatagcaggtggaacagggataactccagtttatcaagtcatgcaggcaattctgaaagatccagaagatgacacagaaatgtatgtggtctatgctaatagaacagaggatgatattttacttaaggaagagcttgattcatgggctgagaaaattccagaaagggttaaagtttggtatgtggttcaagattctattaaagaaggatggaagtacagccttggttttatttcagaagccattttgagagaacatatccctgagccatctcacacaacactggctttggcttgtggaccacctcctatgattcaatttgctgttaatccaaacttggagaagatgggctatgacattaaggattccttattggtgttctaa

SEQ ID NO: 2 - protein, 904 aa, Nicotiana tabacum
MAASVENRQFSHIEAGLSRSFKPRSDSPVRGCNFPPPNSTNFQKKPNSTIFLDYSSSEDDDDDDEKNEYLQMIKKGNSELEPSVHDSRDEGTADNWIERNFSLIRLTGKHPFNSEPPLNRLMHHGFITPVPLHYVRNHGPVPKGTWDDWTVEVTGLVKRPMKFTMDQLVNEFPSRELPVTLVCAGNRRKEQNMVKQTIGFNWGAAAVSTTVWRGVPLRALLKRCGVFSKNKGALNVCFEGADVLPGGGGSKYGTSIKKEFAMDPARDIIIAYMQNGEKLAPDHGFPVRMIIPGFIGGRMVKWIKRIIVTTQESDSYYHFKDNRVLPPHVDAELANTEAWWYKPEYIINELNINSVITTPCHEEILPINAWTTQRPYTLRGYSYSGGGKKVTRVEVTLDGGETWQVCTLDHPEKPTKYGKYWCWCFWSLEVEVLDLLSAKEIAVRAWDETLNTQPEKLIWNVMGMMNNCWFRVKMNVCKPHKGEIGIVFEHPTQPGNQSGGWMAKERHLEISAEAPPTLKKSISTPFMNTASKMYSMSEVRKHSSADSAWIIVHGHIYDATRFLKDHPGGSDSILINAGTDCTEEFDAIHSDKAKKLLEEFRIGELITTGYTSDSPGNSVHGSSSFSSFLAPIKELVPAQRSVALIPREKIPCKLIDKQSISPDVRKFRFALPSEDQVLGLPVGKHIFLCAVIDDKLCMRAYTPTSTIDEVGYFELVVKIYFKGIHPKFPNGGQMSQYLDSLQLGSFLDVKGPLGHIEYQGKGNFLVHGKQKFAKKLAMIAGGTGITPVYQVMQAILKDPEDDTEMYVVYANRTEDDILLKEELDSWAEKIPERVKVWYVVQDSIKEGWKYSLGFISEAILREHIPEPSHTTLALACGPPPMIQFAVNPNLEKMGYDIKDSLLVF

SEQ ID NO: 3 - DNA, 2715 bp, Nicotiana tabacum
  CDS (1)..(2715)
atggcggcatctgtcgaaaacaggcagttcagtcacctagaagccggtttatcccggtctttcaagccccggtctgattccccggttcgtggctgcaacttcccttcgcccaacagtactaatttccaaaagaaaccaaattccaccatttaccttgattactcgtcgagtgaagacgacgatgatgatgacgaaaaaaatgagtaccttcaaatgattaaaaaagggaattcagagttagagccatctgttcatgacactagggacgaaggtaccgctgataattggattgaacgcaacttttccatgattcgtctcaccggaaagcatccatttaactccgaaccaccgttgaaccggctcatgcaccacggctttatcacaccggtcccacttcattacgttcgtaaccatggaccggttcccaagggcacgtgggatgactggaccgtggaagtcacgggactagtgaagcgtcctatgaaattcacaatggaccagttggttaacgaattcccttgtagagaattgcccgttacgcttgtttgtgctggcaatcgaaggaaagaacagaacatggttaaacaaaccattggtttcaactggggcgccgctgccgtttcaacaacgatatggcgcggggtacccctccgcgctttgctaaaacggtgcggtgtttttagcaagaataaaggggcgcttaatgtttgcttcgaaggagctgatgtgttgcccggaggtggtggttcaaagtatggaaccagcattaagaaggaatttgcaatggatccagcacgagatatcatcgtagcctacatgcagaacggagaaaaattggcacccgaccacgggtttccagtacgaatgataattccaggattcattggaggaagaatggtgaaatggataaagaggattatagtcaccacccaagaatcagacagctattatcatttcaaggacaatagagttcttcctccccatgttgatgctgaacttgcaaataccgaagcatggtggtacaagccagagtatatcatcaatgagcttaatattaactctgtcattacgacgccgtgtcatgaagaaattttgccaattaacgcctggacgactcagcgaccttacacgttgaggggctattcttattctggcggagggaaaaaagtaacgcgagtagaagtgacgttggatggaggagaaacatggcaagttagcacactagatcacccagagaagcccaccaaatatggcaagtactggtgttggtgcttttggtcactcgaggttgaggtgttagacttgctcagtgctaaagaaattgctgttcgagcttgggatgagaccctcaatactcaacccgagaagcttatttggaacgtcatgggaatgatgaataattgctggttccgagtaaagatgaatgtgtgcaagcctcacaagggagagattggaatagtgtttgagcatccgactcaacctggaaaccaatcaggtggatggatggcgaaggagagacatttggagatatcagcagaggcacctcaaacactaaagaagagtatctcaactccattcatgaacacagcttccaagatgtactccatgtccgaggtcaggaaacacagctctgctgactctgcttggatcatagtccatggtcatatctatgacgccacgcgtttcttgaaagatcaccctggtgggactgacagcattctcatcaatgctggcactgattgcactgaggaatttgatgcaattcattctgataaggctaagaagctcttggaggatttcaggattggtgaactcataactactggttacacctctgactctcctggcaactccgtgcacggatcttcttccttcagcagctttctagcacctattaaggaacttgttccagcgcagaggagtgtggccctaattccaagagagaaaatcccatgcaaactcatcgacaagcaatccatctcccatgatgttaggaaatttcgatttgcattgccctctgaggatcaagtcttgggcttgcctgttggaaaacatatcttcctctgtgccgttattgacgataagctctgcatgcgcgcttacacgcctactagcacgatcgatgaggtggggtacttcgagttggttgtcaagatatacttcaaaggaattcaccctaaattccccaatggagggcaaatgtcacagtatcttgattctatgccgttagggtcatttctcgacgtgaaaggtccattaggtcacattgaataccaaggaaagggaaatttcttagttcatggcaaacagaagtttgccaagaagttggccatgatagcaggtggaacaggaataactccagtgtatcaagtcatgcaggcaattctgaaagatccagaagatgacacagaaatgtatgtggtgtatgctaacagaacagaggatgatattttacttaaggaagagcttgattcatgggctgagaaaattccagagagggttaaagtttggtatgtggttcaggattctattaaagaaggatggaagtacagcattggttttattacagaagccattttgagagaacatatccctgagccatctcacacaacactggctttggcttgtggaccacctcctatgattcaatttgctgttaatccaaacttggagaagatgggctatgacattaaggattccttattggtgttctaa

SEQ ID NO: 4 - protein, 904 aa, Nicotiana tabacum
MAASVENRQFSHLEAGLSRSFKPRSDSPVRGCNFPSPNSTNFQKKPNSTIYLDYSSSEDDDDDDEKNEYLQMIKKGNSELEPSVHDTRDEGTADNWIERNFSMIRLTGKHPFNSEPPLNRLMHHGFITPVPLHYVRNHGPVPKGTWDDWTVEVTGLVKRPMKFTMDQLVNEFPCRELPVTLVCAGNRRKEQNMVKQTIGFNWGAAAVSTTIWRGVPLRALLKRCGVFSKNKGALNVCFEGADVLPGGGGSKYGTSIKKEFAMDPARDIIVAYMQNGEKLAPDHGFPVRMIIPGFIGGRMVKWIKRIIVTTQESDSYYHFKDNRVLPPHVDAELANTEAWWYKPEYIINELNINSVITTPCHEEILPINAWTTQRPYTLRGYSYSGGGKKVTRVEVTLDGGETWQVSTLDHPEKPTKYGKYWCWCFWSLEVEVLDLLSAKEIAVRAWDETLNTQPEKLIWNVMGMMNNCWFRVKMNVCKPHKGEIGIVFEHPTQPGNQSGGWMAKERHLEISAEAPQTLKKSISTPFMNTASKMYSMSEVRKHSSADSAWIIVHGHIYDATRFLKDHPGGTDSILINAGTDCTEEFDAIHSDKAKKLLEDFRIGELITTGYTSDSPGNSVHGSSSFSSFLAPIKELVPAQRSVALIPREKIPCKLIDKQSISHDVRKFRFALPSEDQVLGLPVGKHIFLCAVIDDKLCMRAYTPTSTIDEVGYFELVVKIYFKGIHPKFPNGGQMSQYLDSMPLGSFLDVKGPLGHIEYQGKGNFLVHGKQKFAKKLAMIAGGTGITPVYQVMQAILKDPEDDTEMYVVYANRTEDDILLKEELDSWAEKIPERVKVWYVVQDSIKEGWKYSIGFITEAILREHIPEPSHTTLALACGPPPMIQFAVNPNLEKMGYDIKDSLLVF

SEQ ID NO: 5 - protein, 904 aa, Nicotiana tabacum
MAASVENRQFSHIEAGLSRSFKPRSDSPVRGCNFPPPNSTNFQKKPNSTIFLDYSSSEDDDDDDEKNEYLQMIKKGNSELEPSVHDSRDEGTADNWIERNFSLIRLTGKHPFNSEPPLNRLMHHGFITPVPLHYVRNHGPVPKGTWDDWTVEVTGLVKRPMKFTMDQLVNEFPSRELPVTLVCAGNRRKEQNMVKQTIGFNWGAAAVSTTVWRGVPLRALLKRCGVFSKNKGALNVCFEGADVLPGGGGSKYGTSIKKEFAMDPARDIIIAYMQNGEKLAPDHGFPVRMIIPGFIGGRMVKWIKRIIVTTQESDSYYHFKDNRVLPPHVDAELANTEAWWYKPEYIINELNINSVITTPCHEEILPINAWTTQRPYTLRGYSYSGGGKKVTRVEVTLDGGETWQVCTLDHPEKPTKYGKYWCWCFWSLEVEVLDLLSAKEIAVRAWDETLNTQPEKLIWNVMGMMNNCWFRVKMNVCKPHKGEIGIVFEHPTQPGNQSGGWMAKERHLEISAEAPPTLKKSISTLFMNTASKMYSMSEVRKHSSADSAWIIVHGHIYDATRFLKDHPGGSDSILINAGTDCTEEFDAIHSDKAKKLLEEFRIGELITTGYTSDSPGNSVHGSSSFSSFLAPIKELVPAQRSVALIPREKIPCKLIDKQSISPDVRKFRFALPSEDQVLGLPVGKHIFLCAVIDDKLCMRAYTPTSTIDEVGYFELVVKIYFKGIHPKFPNGGQMSQYLDSLQLGSFLDVKGPLGHIEYQGKGNFLVHGKQKFAKKLAMIAGGTGITPVYQVMQAILKDPEDDTEMYVVYANRTEDDILLKEELDSWAEKIPERVKVWYVVQDSIKEGWKYSLGFISEAILREHIPEPSHTTLALACGPPPMIQFAVNPNLEKMGYDIKDSLLVF

SEQ ID NO: 6 - protein, 904 aa, Nicotiana tabacum
MAASVENRQFSHLEAGLSRSFKPRSDSPVRGCNFPSPNSTNFQKKPNSTIYLDYSSSEDDDDDDEKNEYLQMIKKGNSELEPSVHDTRDEGTADNWIERNFSMIRLTGKHPFNSEPPLNRLMHHGFITPVPLHYVRNHGPVPKGTWDDWTVEVTGLVKRPMKFTMDQLVNEFPCRELPVTLVCAGNRRKEQNMVKQTIGFNWGAAAVSTTIWRGVPLRALLKRCGVFSKNKGALNVCFEGADVLPGGGGSKYGTSIKKEFAMDPARDIIVAYMQNGEKLAPDHGFPVRMIIPGFIGGRMVKWIKRIIVTTQESDSYYHFKDNRVLPPHVDAELANTEAWWYKPEYIINELNINSVITTPCHEEILPINAWTTQRPYTLRGYSYSGGGKKVTRVEVTLDGGETWQVSTLDHPEKPTKYGKYWCWCFWSLEVEVLDLLSAKEIAVRAWDETLNTQPEKLIWNVMGMMNNCWFRVKMNVCKPHKGEIGIVFEHPTQPGNQSGGWMAKERHLEISAEAPQTLKKSISTLFMNTASKMYSMSEVRKHSSADSAWIIVHGHIYDATRFLKDHPGGTDSILINAGTDCTEEFDAIHSDKAKKLLEDFRIGELITTGYTSDSPGNSVHGSSSFSSFLAPIKELVPAQRSVALIPREKIPCKLIDKQSISHDVRKFRFALPSEDQVLGLPVGKHIFLCAVIDDKLCMRAYTPTSTIDEVGYFELVVKIYFKGIHPKFPNGGQMSQYLDSMPLGSFLDVKGPLGHIEYQGKGNFLVHGKQKFAKKLAMIAGGTGITPVYQVMQAILKDPEDDTEMYVVYANRTEDDILLKEELDSWAEKIPERVKVWYVVQDSIKEGWKYSIGFITEAILREHIPEPSHTTLALACGPPPMIQFAVNPNLEKMGYDIKDSLLVF

SEQ ID NO: 7 - protein, 904 aa, Nicotiana tabacum
MAASVENRQFSHIEAGLSRSFKPRSDSPVRGCNFPPPNSTNFQKKPNSTIFLDYSSSEDDDDDDEKNEYLQMIKKGNSELEPSVHDSRDEGTADNWIERNFSLIRLTGKHPFNSEPPLNRLMHHGFITPVPLHYVRNHGPVPKGTWDDWTVEVTGLVKRPMKFTMDQLVNEFPSRELPVTLVCAGNRRKEQNMVKQTIGFNWGAAAVSTTVWRGVPLRALLKRCGVFSKNKGALNVCFEGADVLPGGGGSKYGTSIKKEFAMDPARDIIIAYMQNGEKLAPDHGFPVRMIIPGFIGGRMVKWIKRIIVTTQESDSYYHFKDNRVLPPHVDAELANTEAWWYKPEYIINELNINSVITTPCHEEILPINAWTTQRPYTLRGYSYSGGGKKVTRVEVTLDGGETWQVCTLDHPEKPTKYGKYWCWCFWSLEVEVLDLLSAKEIAVRAWDETLNTQPEKLIWNVMGMMNNCWFRVKMNVCKPHKGEIGIVFEHPTQPGNQSGGWMAKERHLEISAEAPPTLKKSISTSFMNTASKMYSMSEVRKHSSADSAWIIVHGHIYDATRFLKDHPGGSDSILINAGTDCTEEFDAIHSDKAKKLLEEFRIGELITTGYTSDSPGNSVHGSSSFSSFLAPIKELVPAQRSVALIPREKIPCKLIDKQSISPDVRKFRFALPSEDQVLGLPVGKHIFLCAVIDDKLCMRAYTPTSTIDEVGYFELVVKIYFKGIHPKFPNGGQMSQYLDSLQLGSFLDVKGPLGHIEYQGKGNFLVHGKQKFAKKLAMIAGGTGITPVYQVMQAILKDPEDDTEMYVVYANRTEDDILLKEELDSWAEKIPERVKVWYVVQDSIKEGWKYSLGFISEAILREHIPEPSHTTLALACGPPPMIQFAVNPNLEKMGYDIKDSLLVF

SEQ ID NO: 8 - protein, 904 aa, Nicotiana tabacum
MAASVENRQFSHLEAGLSRSFKPRSDSPVRGCNFPSPNSTNFQKKPNSTIYLDYSSSEDDDDDDEKNEYLQMIKKGNSELEPSVHDTRDEGTADNWIERNFSMIRLTGKHPFNSEPPLNRLMHHGFITPVPLHYVRNHGPVPKGTWDDWTVEVTGLVKRPMKFTMDQLVNEFPCRELPVTLVCAGNRRKEQNMVKQTIGFNWGAAAVSTTIWRGVPLRALLKRCGVFSKNKGALNVCFEGADVLPGGGGSKYGTSIKKEFAMDPARDIIVAYMQNGEKLAPDHGFPVRMIIPGFIGGRMVKWIKRIIVTTQESDSYYHFKDNRVLPPHVDAELANTEAWWYKPEYIINELNINSVITTPCHEEILPINAWTTQRPYTLRGYSYSGGGKKVTRVEVTLDGGETWQVSTLDHPEKPTKYGKYWCWCFWSLEVEVLDLLSAKEIAVRAWDETLNTQPEKLIWNVMGMMNNCWFRVKMNVCKPHKGEIGIVFEHPTQPGNQSGGWMAKERHLEISAEAPQTLKKSISTSFMNTASKMYSMSEVRKHSSADSAWIIVHGHIYDATRFLKDHPGGTDSILINAGTDCTEEFDAIHSDKAKKLLEDFRIGELITTGYTSDSPGNSVHGSSSFSSFLAPIKELVPAQRSVALIPREKIPCKLIDKQSISHDVRKFRFALPSEDQVLGLPVGKHIFLCAVIDDKLCMRAYTPTSTIDEVGYFELVVKIYFKGIHPKFPNGGQMSQYLDSMPLGSFLDVKGPLGHIEYQGKGNFLVHGKQKFAKKLAMIAGGTGITPVYQVMQAILKDPEDDTEMYVVYANRTEDDILLKEELDSWAEKIPERVKVWYVVQDSIKEGWKYSIGFITEAILREHIPEPSHTTLALACGPPPMIQFAVNPNLEKMGYDIKDSLLVF

SEQ ID NO: 9 - DNA, 20 bp, Artificial Sequence
  primer for sequencing Nia2_ex1_2F
accgaagcatggtggtacaa

SEQ ID NO: 10 - DNA, 22 bp, Artificial Sequence
  primer for sequencing Nia2_ex2_3F
ggctattcttattctggcggag

SEQ ID NO: 11 - DNA, 20 bp, Artificial Sequence
  primer for sequencing Nia2_ex3_4R
catcattcccatgacgttcc

SEQ ID NO: 12 - DNA, 21 bp, Artificial Sequence
  primer for sequencing Nia2_ex4_HindIII_R
gctgctgaagcttgaagatcc

SEQ ID NO: 13 - DNA, 24 bp, Artificial Sequence
  primer NRs_TMF
caggattggtgaactcataactac

SEQ ID NO: 14 - DNA, 18 bp, Artificial Sequence
  primer NRs_TMR
ctctgcgctggaacaagt

SEQ ID NO: 15 - DNA, 20 bp, Artificial Sequence
  probe NRs_wt_WGB
gatcttcttccttcagcagc

SEQ ID NO: 16 - DNA, 20 bp, Artificial Sequence
  probe NRs_tg_MGB
ggatcttcaagcttcagcag

SEQ ID NO: 17 - DNA, 20 bp, Artificial Sequence
  primer elfa_v2_TMF
ctaagggtgctgccagcttt

SEQ ID NO: 18 - DNA, 22 bp, Artificial Sequence
  primer elfa_v2_TMR
gtcaagcactggagcatatcca

SEQ ID NO: 19 - DNA, 26 bp, Artificial Sequence
  probe elfa_v2_TMP
atcatgaaccatccaggacagattgg

SEQ ID NO: 20 - DNA, 24 bp, Artificial Sequence
  primer NIA1_hinge1_F2
ttaggtgaaataacgctcttacac

SEQ ID NO: 21 - DNA, 24 bp, Artificial Sequence
  primer NIA1_hinge1_R2
cctaattggagagaatcaaggtat

SEQ ID NO: 22 - DNA, 24 bp, Artificial Sequence
  primer NIA2_hinge1_F2
attgtgctatgttgcaatgttcag

SEQ ID NO: 23 - DNA, 19 bp, Artificial Sequence
  primer NIA2_hinge1_R1
ggaagaagatccgtgcacg

SEQ ID NO: 24 - DNA, 2724 bp, Nicotiana tabacum
  CDS (4)..(2718)
catatggcggcatctgtcgaaaacaggcagttcagtcacctagaagccggtttatcccggtctttcaagccccggtctgattccccggttcgtggctgcaacttcccttcgcccaacagtactaatttccaaaagaaaccaaattccaccatttaccttgattactcgtcgagtgaagacgacgatgatgatgacgaaaaaaatgagtaccttcaaatgattaaaaaagggaattcagagttagagccatctgttcatgacactagggacgaaggtaccgctgataattggattgaacgcaacttttccatgattcgtctcaccggaaagcatccatttaactccgaaccaccgttgaaccggctcatgcaccacggctttatcacaccggtcccacttcattacgttcgtaaccatggaccggttcccaagggcacgtgggatgactggaccgtggaagtcacgggactagtgaagcgtcctatgaaattcacaatggaccagttggttaacgaattcccttgtagagaattgcccgttacgcttgtttgtgctggcaatcgaaggaaagaacagaacatggttaaacaaaccattggtttcaactggggcgccgctgccgtttcaacaacgatatggcgcggggtacccctccgcgctttgctaaaacggtgcggtgtttttagcaagaataaaggggcgcttaatgtttgcttcgaaggagctgatgtgttgcccggaggtggtggttcaaagtatggaaccagcattaagaaggaatttgcaatggatccagcacgagatatcatcgtagcctacatgcagaacggagaaaaattggcacccgaccacgggtttccagtacgaatgataattccaggattcattggaggaagaatggtgaaatggataaagaggattatagtcaccacccaagaatcagacagctattatcatttcaaggacaatagagttcttcctccccatgttgatgctgaacttgcaaataccgaagcatggtggtacaagccagagtatatcatcaatgagcttaatattaactctgtcattacgacgccgtgtcatgaagaaattttgccaattaacgcctggacgactcagcgaccttacacgttgaggggctattcttattctggcggagggaaaaaagtaacgcgagtagaagtgacgttggatggaggagaaacatggcaagttagcacactagatcacccagagaagcccaccaaatatggcaagtactggtgttggtgcttttggtcactcgaggttgaggtgttagacttgctcagtgctaaagaaattgctgttcgagcttgggatgagaccctcaatactcaacccgagaagcttatttggaacgtcatgggaatgatgaataattgctggttccgagtaaagatgaatgtgtgcaagcctcacaagggagagattggaatagtgtttgagcatccgactcaacctggaaaccaatcaggtggatggatggcgaaggagagacatttggagatatcagcagaggcacctcaaacactaaagaagagtatcgatactccattcatgaacacagcttccaagatgtactccatgtccgaggtcaggaaacacagctctgctgactctgcttggatcatagtccatggtcatatctatgacgccacgcgtttcttgaaagatcaccctggtgggactgacagcattctcatcaatgctggcactgattgcactgaggaatttgatgcaattcattctgataaggctaagaagctcttggaggatttcaggattggtgaactcataactactggttacacctctgactctcctggcaactccgtgcacggatcttcaagcttcagcagctttctagcacctattaaggaacttgttccagcgcagaggagtgtggccctaattccaagagagaaaatcccatgcaaactcatcgacaagcaatccatctcccatgatgttaggaaatttcgatttgcattgccctctgaggatcaagtcttgggcttgcctgttggaaaacatatcttcctctgtgccgttattgacgataagctctgcatgcgcgcttacacgcctactagcacgatcgatgaggtggggtacttcgagttggttgtcaagatatacttcaaaggaattcaccctaaattccccaatggagggcaaatgtcacagtatcttgattctatgccgttagggtcatttctcgacgtgaaaggtccattaggtcacattgaataccaaggaaagggaaatttcttagttcatggcaaacagaagtttgccaagaagttggccatgatagcaggtggaacaggaataactccagtgtatcaagtcatgcaggcaattctgaaagatccagaagatgacacagaaatgtatgtggtgtatgctaacagaacagaggatgatattttacttaaggaagagcttgattcatgggctgagaaaattccagagagggttaaagtttggtatgtggttcaggattctattaaagaaggatggaagtacagcattggttttattacagaagccattttgagagaacatatccctgagccatctcacacaacactggctttggcttgtggaccacctcctatgattcaatttgctgttaatccaaacttggagaagatgggctatgacattaaggattccttattggtgttctaagtcgac

SEQ ID NO: 25 - DNA, 2724 bp, Nicotiana tabacum
  CDS (4)..(2718)
catatggcggcatctgtcgaaaacaggcagttcagtcacctagaagccggtttatcccggtctttcaagccccggtctgattccccggttcgtggctgcaacttcccttcgcccaacagtactaatttccaaaagaaaccaaattccaccatttaccttgattactcgtcgagtgaagacgacgatgatgatgacgaaaaaaatgagtaccttcaaatgattaaaaaagggaattcagagttagagccatctgttcatgacactagggacgaaggtaccgctgataattggattgaacgcaacttttccatgattcgtctcaccggaaagcatccatttaactccgaaccaccgttgaaccggctcatgcaccacggctttatcacaccggtcccacttcattacgttcgtaaccatggaccggttcccaagggcacgtgggatgactggaccgtggaagtcacgggactagtgaagcgtcctatgaaattcacaatggaccagttggttaacgaattcccttgtagagaattgcccgttacgcttgtttgtgctggcaatcgaaggaaagaacagaacatggttaaacaaaccattggtttcaactggggcgccgctgccgtttcaacaacgatatggcgcggggtacccctccgcgctttgctaaaacggtgcggtgtttttagcaagaataaaggggcgcttaatgtttgcttcgaaggagctgatgtgttgcccggaggtggtggttcaaagtatggaaccagcattaagaaggaatttgcaatggatccagcacgagatatcatcgtagcctacatgcagaacggagaaaaattggcacccgaccacgggtttccagtacgaatgataattccaggattcattggaggaagaatggtgaaatggataaagaggattatagtcaccacccaagaatcagacagctattatcatttcaaggacaatagagttcttcctccccatgttgatgctgaacttgcaaataccgaagcatggtggtacaagccagagtatatcatcaatgagcttaatattaactctgtcattacgacgccgtgtcatgaagaaattttgccaattaacgcctggacgactcagcgaccttacacgttgaggggctattcttattctggcggagggaaaaaagtaacgcgagtagaagtgacgttggatggaggagaaacatggcaagttagcacactagatcacccagagaagcccaccaaatatggcaagtactggtgttggtgcttttggtcactcgaggttgaggtgttagacttgctcagtgctaaagaaattgctgttcgagcttgggatgagaccctcaatactcaacccgagaagcttatttggaacgtcatgggaatgatgaataattgctggttccgagtaaagatgaatgtgtgcaagcctcacaagggagagattggaatagtgtttgagcatccgactcaacctggaaaccaatcaggtggatggatggcgaaggagagacatttggagatatcagcagaggcacctcaaacactaaagaagagtatctcaactccattcatgaacacagcttccaagatgtactccatgtccgaggtcaggaaacacagctctgctgactctgcttggatcatagtccatggtcatatctatgacgccacgcgtttcttgaaagatcaccctggtgggactgacagcattctcatcaatgctggcactgattgcactgaggaatttgatgcaattcattctgataaggctaagaagctcttggaggatttcaggattggtgaactcataactactggttacacctctgactctcctggcaactccgtgcacggatcttcaagcttcagcagctttctagcacctattaaggaacttgttccagcgcagaggagtgtggccctaattccaagagagaaaatcccatgcaaactcatcgacaagcaatccatctcccatgatgttaggaaatttcgatttgcattgccctctgaggatcaagtcttgggcttgcctgttggaaaacatatcttcctctgtgccgttattgacgataagctctgcatgcgcgcttacacgcctactagcacgatcgatgaggtggggtacttcgagttggttgtcaagatatacttcaaaggaattcaccctaaattccccaatggagggcaaatgtcacagtatcttgattctatgccgttagggtcatttctcgacgtgaaaggtccattaggtcacattgaataccaaggaaagggaaatttcttagttcatggcaaacagaagtttgccaagaagttggccatgatagcaggtggaacaggaataactccagtgtatcaagtcatgcaggcaattctgaaagatccagaagatgacacagaaatgtatgtggtgtatgctaacagaacagaggatgatattttacttaaggaagagcttgattcatgggctgagaaaattccagagagggttaaagtttggtatgtggttcaggattctattaaagaaggatggaagtacagcattggttttattacagaagccattttgagagaacatatccctgagccatctcacacaacactggctttggcttgtggaccacctcctatgattcaatttgctgttaatccaaacttggagaagatgggctatgacattaaggattccttattggtgttctaagtcgac